European Patent Specification EP 3 275 448 B1, published October 29, 2025. Title: Lipid Nanoparticles Comprising Nucleotide. Applicant: KYOWA HAKKO KIRIN CO., LTD. The sequence listing filed with the application follows.

SEQUENCE LISTING (4 sequences)

SEQ ID NO: 1 - RNA, 21 nt, Artificial Sequence
  Luc siRNA sense
ccgucguauucgugagcaaga

SEQ ID NO: 2 - RNA, 21 nt, Artificial Sequence
  Luc siRNA antisense
uugcucacgaauacgacggug

SEQ ID NO: 3 - DNA, 25 bp, Artificial Sequence
  AF488-HPRT1 siRNA sense
  misc_feature (1)..(23): RNA
  misc_feature (24)..(25): DNA
gccagacuuuguuggauuugaaatt

SEQ ID NO: 4 - RNA, 27 nt, Artificial Sequence
  AF488-HPRT1 siRNA antisense
  modified_base (9)..(9): am
  modified_base (11)..(11): cm
  modified_base (13)..(13): am
  modified_base (15)..(15): cm
  modified_base (17)..(17): am
  modified_base (19)..(19): gm
  modified_base (21)..(21): cm
  modified_base (23)..(23): gm
  modified_base (25)..(25): cm
  modified_base (26)..(27): um
aauuucaaauccaacaaagucuggcuu